European Patent Specification EP 4 143 193 B1, published April 22, 2026. Title: IMIDAZOPYRIMIDINES AS MODULATORS OF IL-17. Applicant: Janssen Biotech, Inc. Goldberg, Steven Martin, Connor Rhorer,Timothy Tanis, Virginia Xue, Xiaohua. Application To Be Assigned. The sequence listing filed with the application follows.

SEQUENCE LISTING (2 sequences)

SEQ ID NO: 1 - protein, 182 aa, artificial
  Human IL17A with a FLAg tag
MATGSRTSLLLAFGLLCLPWLQEGSAGSDYKDDDDKGSGSGSLEVLFQGPGITIPRNPGCPNSEDKNFPRTVMVNLNIHNRNTNTNPKRSSDYYNRSTSPWNLHRNEDPERYPSVIWEAQCRHLGCINADGNVDYHMNSVPIQQEILVLRREPPHCPNSFRLEKILVSVGCTCVTPIVHHVQ

SEQ ID NO: 2 - protein, 323 aa, artificial
  IL17A with a His tag
MKFLVNVALVFMVVYISYIYALRLLDHRALVCSQPGLNCTVKNSTCLDDSWIHPRNLTPSSPKDLQIQLHFAHTQQGDLFPVAHIEWTLQTDASILYLEGAELSVLQLNTNERLCVRFEFLSKLRHHHRRWRFTFSHFVVDPDQEYEVTVHHLPKPIPDGDPNHQSKNFLVPDCEHARMKVTTPCMSSGSLWDPNITVETLEAHQLRVSFTLWNESTHYQILLTSFPHMENHSCFEHMHHIPAPRPEEFHQRSNVTLTLRNLKGCCRHQVQIQPFFSSCLNDCLRHSATVSCPEMPDTPEPIPDYMPLWGSGGHHHHHHHHHH